European Patent Specification EP 3 946 621 B1, published May 21, 2025. Title: MAGE-A4-TCRs. Applicant: GmbH, Medigene Immunotherapies Bluebird bio, Inc. The sequence listing filed with the application follows.

SEQUENCE LISTING (116 sequences)

SEQ ID NO: 1 - protein, 10 aa, Homo sapiens
GVYDGREHTV

SEQ ID NO: 2 - protein, 7 aa, Homo sapiens
TSDQSYG

SEQ ID NO: 3 - protein, 8 aa, Homo sapiens
QGSYDEQN

SEQ ID NO: 4 - protein, 14 aa, Homo sapiens
CAMSGDSAGNMLTF

SEQ ID NO: 5 - protein, 5 aa, Homo sapiens
KGHDR

SEQ ID NO: 6 - protein, 6 aa, Homo sapiens
SFDVKD

SEQ ID NO: 7 - protein, 17 aa, Homo sapiens
CATSDWDRSGDKETQYF

SEQ ID NO: 8 - protein, 136 aa, Homo sapiens
MSLSSLLKVVTASLWLGPGIAQKITQTQPGMFVQEKEAVTLDCTYDTSDQSYGLFWYKQPSSGEMIFLIYQGSYDEQNATEGRYSLNFQKARKSANLVISASQLGDSAMYFCAMSGDSAGNMLTFGGGTRLMVKPH

SEQ ID NO: 9 - protein, 135 aa, Homo sapiens
MASLLFFCGAFYLLGTGSMDADVTQTPRNRITKTGKRIMLECSQTKGHDRMYWYRQDPGLGLRLIYYSFDVKDINKGEISDGYSVSRQAQAKFSLSLESAIPNQTALYFCATSDWDRSGDKETQYFGPGTRLLVL

SEQ ID NO: 10 - protein, 276 aa, Artificial Sequence
  with mininmal murinized constant region
MSLSSLLKVVTASLWLGPGIAQKITQTQPGMFVQEKEAVTLDCTYDTSDQSYGLFWYKQPSSGEMIFLIYQGSYDEQNATEGRYSLNFQKARKSANLVISASQLGDSAMYFCAMSGDSAGNMLTFGGGTRLMVKPHIQNPDPAVYQLRDSKSSDKSVCLFTDFDSQTNVSQSKDSDVYITDKTVLDMRSMDFKSNSAVAWSNKSDFACANAFNNSIIPEDTFFPSSDVPCDVKLVEKSFETDTNLNFQNLSVIGFRILLLKVAGFNLLMTLRLWSS

SEQ ID NO: 11 - protein, 312 aa, Artificial Sequence
  with minimal murinized constant region
MASLLFFCGAFYLLGTGSMDADVTQTPRNRITKTGKRIMLECSQTKGHDRMYWYRQDPGLGLRLIYYSFDVKDINKGEISDGYSVSRQAQAKFSLSLESAIPNQTALYFCATSDWDRSGDKETQYFGPGTRLLVLEDLNKVFPPEVAVFEPSKAEIAHTQKATLVCLATGFFPDHVELSWWVNGKEVHSGVSTDPQPLKEQPALNDSRYCLSSRLRVSATFWQNPRNHFRCQVQFYGLSENDEWTQDRAKPVTQIVSAEAWGRADCGITSASYHQGVLSATILYEILLGKATLYAVLVSALVLMAMVKRKDF

SEQ ID NO: 12 - protein, 7 aa, Homo sapiens
TSDPSYG

SEQ ID NO: 13 - protein, 8 aa, Homo sapiens
QGSYDQQN

SEQ ID NO: 14 - protein, 15 aa, Homo sapiens
CAMSGGYTGGFKTIF

SEQ ID NO: 15 - protein, 5 aa, Homo sapiens
SGDLS

SEQ ID NO: 16 - protein, 6 aa, Homo sapiens
YYNGEE

SEQ ID NO: 17 - protein, 13 aa, Homo sapiens
CASSGGDGDEQFF

SEQ ID NO: 18 - protein, 137 aa, Homo sapiens
MSLSSLLKVVTASLWLGPGIAQKITQTQPGMFVQEKEAVTLDCTYDTSDPSYGLFWYKQPSSGEMIFLIYQGSYDQQNATEGRYSLNFQKARKSANLVISASQLGDSAMYFCAMSGGYTGGFKTIFGAGTRLFVKAN

SEQ ID NO: 19 - protein, 131 aa, Homo sapiens
MGFRLLCCVAFCLLGAGPVDSGVTQTPKHLITATGQRVTLRCSPRSGDLSVYWYQQSLDQGLQFLIQYYNGEERAKGNILERFSAQQFPDLHSELNLSSLELGDSALYFCASSGGDGDEQFFGPGTRLTVL

SEQ ID NO: 20 - protein, 277 aa, Artificial Sequence
  with minimal  murinized constant region
MSLSSLLKVVTASLWLGPGIAQKITQTQPGMFVQEKEAVTLDCTYDTSDPSYGLFWYKQPSSGEMIFLIYQGSYDQQNATEGRYSLNFQKARKSANLVISASQLGDSAMYFCAMSGGYTGGFKTIFGAGTRLFVKANIQNPDPAVYQLRDSKSSDKSVCLFTDFDSQTNVSQSKDSDVYITDKTVLDMRSMDFKSNSAVAWSNKSDFACANAFNNSIIPEDTFFPSSDVPCDVKLVEKSFETDTNLNFQNLSVIGFRILLLKVAGFNLLMTLRLWSS

SEQ ID NO: 21 - protein, 310 aa, Artificial Sequence
  with minimal murinized constant region
MGFRLLCCVAFCLLGAGPVDSGVTQTPKHLITATGQRVTLRCSPRSGDLSVYWYQQSLDQGLQFLIQYYNGEERAKGNILERFSAQQFPDLHSELNLSSLELGDSALYFCASSGGDGDEQFFGPGTRLTVLEDLKNVFPPEVAVFEPSKAEIAHTQKATLVCLATGFYPDHVELSWWVNGKEVHSGVSTDPQPLKEQPALNDSRYCLSSRLRVSATFWQNPRNHFRCQVQFYGLSENDEWTQDRAKPVTQIVSAEAWGRADCGITSRSYHQGVLSATILYEILLGKATLYAVLVSALVLMAMVKRKDSRG

SEQ ID NO: 22 - protein, 6 aa, Homo sapiens
DSASNY

SEQ ID NO: 23 - protein, 7 aa, Homo sapiens
IRSNVGE

SEQ ID NO: 24 - protein, 14 aa, Homo sapiens
CAASRGTGFQKLVF

SEQ ID NO: 25 - protein, 5 aa, Homo sapiens
LGHDT

SEQ ID NO: 26 - protein, 6 aa, Homo sapiens
YNNKEL

SEQ ID NO: 27 - protein, 16 aa, Homo sapiens
CASSQFWDGAGDEQYF

SEQ ID NO: 28 - protein, 133 aa, Homo sapiens
MTSIRAVFIFLWLQLDLVNGENVEQHPSTLSVQEGDSAVIKCTYSDSASNYFPWYKQELGKRPQLIIDIRSNVGEKKDQRIAVTLNKTAKHFSLHITETQPEDSAVYFCAASRGTGFQKLVFGTGTRLLVSPN

SEQ ID NO: 29 - protein, 134 aa, Homo sapiens
MGCRLLCCVVFCLLQAGPLDTAVSQTPKYLVTQMGNDKSIKCEQNLGHDTMYWYKQDSKKFLKIMFSYNNKELIINETVPNRFSPKSPDKAHLNLHINSLELGDSAVYFCASSQFWDGAGDEQYFGPGTRLTVT

SEQ ID NO: 30 - protein, 273 aa, Artificial Sequence
  with minimal murinized constant region
MTSIRAVFIFLWLQLDLVNGENVEQHPSTLSVQEGDSAVIKCTYSDSASNYFPWYKQELGKRPQLIIDIRSNVGEKKDQRIAVTLNKTAKHFSLHITETQPEDSAVYFCAASRGTGFQKLVFGTGTRLLVSPNIQNPDPAVYQLRDSKSSDKSVCLFTDFDSQTNVSQSKDSDVYITDKTVLDMRSMDFKSNSAVAWSNKSDFACANAFNNSIIPEDTFFPSSDVPCDVKLVEKSFETDTNLNFQNLSVIGFRILLLKVAGFNLLMTLRLWSS

SEQ ID NO: 31 - protein, 311 aa, Artificial Sequence
  with minimal murinized constant region
MGCRLLCCVVFCLLQAGPLDTAVSQTPKYLVTQMGNDKSIKCEQNLGHDTMYWYKQDSKKFLKIMFSYNNKELIINETVPNRFSPKSPDKAHLNLHINSLELGDSAVYFCASSQFWDGAGDEQYFGPGTRLTVTEDLNKVFPPEVAVFEPSKAEIAHTQKATLVCLATGFFPDHVELSWWVNGKEVHSGVSTDPQPLKEQPALNDSRYCLSSRLRVSATFWQNPRNHFRCQVQFYGLSENDEWTQDRAKPVTQIVSAEAWGRADCGITSASYHQGVLSATILYEILLGKATLYAVLVSALVLMAMVKRKDF

SEQ ID NO: 32 - DNA, 21 bp, Artificial Sequence
  Codon optimized
accagcgatcagagctacggc

SEQ ID NO: 33 - DNA, 24 bp, Artificial Sequence
  codon optimized
cagggcagctacgacgagcagaat

SEQ ID NO: 34 - DNA, 42 bp, Artificial Sequence
  codon optimized
tgtgccatgagcggcgatagcgccggcaacatgcttacattt

SEQ ID NO: 35 - DNA, 15 bp, Artificial Sequence
  codon optimized
aagggccacgaccgg

SEQ ID NO: 36 - DNA, 18 bp, Artificial Sequence
  codon optimized
agcttcgacgtgaaggac

SEQ ID NO: 37 - DNA, 51 bp, Artificial Sequence
  codon optimized
tgcgccaccagcgactgggatagaagcggcgacaaagagacacagtacttc

SEQ ID NO: 38 - DNA, 831 bp, Artificial Sequence
  with minimal murinized constant region;  codon optimized
atgagcctgagcagcctgctgaaggtcgtgacagcctctctgtggctcggacctggaatcgcccagaagatcacccagacacagcccggcatgttcgtgcaagagaaagaagccgtgacactggactgcacctacgacaccagcgatcagagctacggcctgttctggtacaagcagcctagcagcggcgagatgatcttcctgatctaccagggcagctacgacgagcagaatgccaccgagggcagatacagcctgaacttccagaaggcccggaagtccgccaacctggtcatttctgcttctcagctgggcgacagcgccatgtacttttgtgccatgagcggcgatagcgccggcaacatgcttacatttggcggcggaacccggctgatggtcaagccccatattcagaaccccgatcctgccgtgtaccagctgagagacagcaagagcagcgacaagagcgtgtgtctgttcaccgacttcgacagccagaccaacgtgtcccagagcaaggacagcgacgtgtacatcaccgacaagaccgtgctggacatgcggagcatggacttcaagagcaacagcgccgtggcctggtccaacaagagcgatttcgcctgcgccaacgccttcaacaatagcattatccccgaggacacattcttccccagctccgatgtgccctgcgacgtgaagctggtggaaaagagcttcgagacagacaccaacctgaacttccagaacctgagcgtgatcggcttcagaatcctgctgctgaaggtggccggcttcaatctgctgatgaccctgagactgtggtccagctga

SEQ ID NO: 39 - DNA, 939 bp, Artificial Sequence
  with minimal murinized constant region; codon optimized
atggccagcctgctgttcttctgcggcgccttttatctgctcggcaccggctctatggacgccgacgttacacagacccctcggaacagaatcaccaagaccggcaagcggatcatgctggaatgcagccagaccaagggccacgaccggatgtactggtacagacaggaccctggcctgggcctgagactgatctactacagcttcgacgtgaaggacatcaacaagggcgagatcagcgacggctacagcgtgtcaagacaggctcaggccaagttcagcctgtctctggaaagcgctatccccaaccagacagccctgtacttctgcgccaccagcgactgggatagaagcggcgacaaagagacacagtacttcggccctggcaccagactgctggtgctggaagatctgaacaaggtgttccctccagaggtggccgtgttcgagccttctaaggccgagattgcccacacacagaaagccacactcgtgtgcctggctaccggcttctttcctgaccacgtggaactgtcttggtgggtcaacggcaaagaggtgcacagcggcgtcagcacagatccccagcctctgaaagaacagcccgctctgaacgacagccggtactgtctgagcagcagactgagagtgtccgccacattctggcagaaccccagaaaccacttcagatgccaggtgcagttctacggcctgagcgagaacgatgagtggacccaggatagagccaagcctgtgacacagatcgtgtctgccgaagcctggggcagagccgattgtggaattaccagcgccagctaccatcagggcgtgctgtctgccacaatcctgtacgagatcctgctgggcaaagccactctgtacgccgtgctggtgtctgccctggtgctgatggccatggtcaagagaaaggacttttga

SEQ ID NO: 40 - DNA, 21 bp, Artificial Sequence
  codon optimized
accagcgatcctagctacggc

SEQ ID NO: 41 - DNA, 24 bp, Artificial Sequence
  codon optimized
cagggcagctacgaccagcagaat

SEQ ID NO: 42 - DNA, 45 bp, Artificial Sequence
  codon optimized
tgtgccatgagcggcggctacaccggcggcttcaagacaatcttt

SEQ ID NO: 43 - DNA, 15 bp, Artificial Sequence
  codon optimized
agcggcgacctgagc

SEQ ID NO: 44 - DNA, 18 bp, Artificial Sequence
  codon optimized
tactacaacggcgaggaa

SEQ ID NO: 45 - DNA, 39 bp, Artificial Sequence
  codon optimized
tgtgccagctctggcggagatggcgacgagcagtttttt

SEQ ID NO: 46 - DNA, 834 bp, Artificial Sequence
  with minimal murinized constant region; codon optimized
atgagcctgagcagcctgctgaaggtcgtgacagcctctctgtggctcggacctggaatcgcccagaagatcacccagacacagcccggcatgttcgtgcaagagaaagaagccgtgacactggactgcacctacgacaccagcgatcctagctacggcctgttctggtacaagcagcctagcagcggcgagatgatcttcctgatctaccagggcagctacgaccagcagaatgccaccgagggcagatacagcctgaacttccagaaggcccggaagtccgccaacctggtcatttctgctagccagctgggcgacagcgccatgtacttttgtgccatgagcggcggctacaccggcggcttcaagacaatctttggcgccggaaccagactgttcgtgaaggccaatattcagaaccccgatcctgccgtgtaccagctgagagacagcaagagcagcgacaagagcgtgtgtctgttcaccgacttcgacagccagaccaacgtgtcccagagcaaggacagcgacgtgtacatcaccgacaagaccgtgctggacatgcggagcatggacttcaagagcaacagcgccgtggcctggtccaacaagagcgatttcgcctgcgccaacgccttcaacaatagcattatccccgaggacacattcttccccagctccgatgtgccctgcgacgtgaagctggtggaaaagagcttcgagacagacaccaacctgaacttccagaacctgagcgtgatcggcttcagaatcctgctgctgaaggtggccggcttcaatctgctgatgaccctgagactgtggtccagctga

SEQ ID NO: 47 - DNA, 933 bp, Artificial Sequence
  with minimal murinized constant region; codon optimized
atgggcttcagactgctgtgctgcgtggccttttgtctgcttggagccggacctgtggatagcggcgttacccagacacctaagcacctgatcacagccacaggccagcgcgtgaccctgagatgttctcctagaagcggcgacctgagcgtgtactggtatcagcagtctctggaccagggcctgcagttcctgatccagtactacaacggcgaggaaagagccaagggcaacatcctggaacggttcagcgcccagcagttcccagatctgcacagcgagctgaacctgagcagcctggaactgggagatagcgccctgtacttctgtgccagctctggcggagatggcgacgagcagttttttggccctggcaccagactgaccgtgctggaggacctgaagaacgtgttccctccggaggtggccgtgttcgagcccagcaaagccgagatcgcgcacacccagaaggccaccctggtgtgcctggccaccggcttctaccccgaccacgtggagctgagctggtgggtgaacggcaaggaggtgcacagcggcgtgagcaccgacccccagcccctgaaggagcagcccgccctgaacgacagccgctactgcctgagcagccgcctgcgcgtgagcgccaccttctggcagaacccccgcaaccacttccgctgccaggtgcagttctacggcctgagcgagaacgacgagtggacccaggaccgcgccaagcccgtgacccagatcgtgagcgccgaggcctggggccgcgccgactgcggcattaccagccgcagctaccatcagggcgtgctgagcgccaccatcctgtacgagatcctgctgggcaaggccaccctgtacgccgtgctggtgagcgccctggtgctgatggcgatggtgaagcgcaaggacagccgcggctga

SEQ ID NO: 48 - DNA, 18 bp, Artificial Sequence
  codon optimized
gacagcgccagcaactac

SEQ ID NO: 49 - DNA, 21 bp, Artificial Sequence
  codon optimized
atccggtccaacgtgggcgag

SEQ ID NO: 50 - DNA, 42 bp, Artificial Sequence
  codon optimized
tgcgctgccagcagaggcaccggcttccagaaactggtgttt

SEQ ID NO: 51 - DNA, 15 bp, Artificial Sequence
  codon optimized
ctgggccacgacacc

SEQ ID NO: 52 - DNA, 18 bp, Artificial Sequence
  codon optimized
tacaacaacaaagagctg

SEQ ID NO: 53 - DNA, 48 bp, Artificial Sequence
  codon optimized
tgtgccagcagccagttctgggatggcgctggcgacgagcagtatttt

SEQ ID NO: 54 - DNA, 822 bp, Artificial Sequence
  with minimal murinized constant region; codon optimized
atgaccagcatccgggccgtgttcatcttcctgtggctgcagctggacctggtcaacggcgagaatgtggaacagcaccccagcacactgagcgtgcaagagggcgattctgccgtgatcaagtgcacctacagcgacagcgccagcaactacttcccctggtacaagcaagagctgggcaaaagaccccagctgatcatcgacatccggtccaacgtgggcgagaagaaggaccagagaatcgccgtgacactgaacaagaccgccaagcacttcagcctgcacatcaccgagacacagcctgaggatagcgccgtgtacttttgcgctgccagcagaggcaccggcttccagaaactggtgtttggcaccggcaccagactgctggtgtccccaaatattcagaaccccgatcctgccgtgtaccagctgagagacagcaagagcagcgacaagagcgtgtgtctgttcaccgacttcgacagccagaccaacgtgtcccagagcaaggacagcgacgtgtacatcaccgacaagaccgtgctggacatgcggagcatggacttcaagagcaacagcgccgtggcctggtccaacaagagcgatttcgcctgcgccaacgccttcaacaatagcattatccccgaggacacattcttccccagctccgatgtgccctgcgacgtgaagctggtggaaaagagcttcgagacagacaccaacctgaacttccagaacctgagcgtgatcggcttcagaatcctgctgctgaaggtggccggcttcaatctgctgatgaccctgagactgtggtccagctga

SEQ ID NO: 55 - DNA, 936 bp, Artificial Sequence
  with minimal murinized constant region; codon optimized
atgggctgcagactgctgtgctgtgtggtgttctgcctgctgcaagccggacctctggatacagccgtgtctcagacccctaagtacctggtcacccagatgggcaacgacaagagcatcaagtgcgagcagaacctgggccacgacaccatgtactggtacaagcaggacagcaagaaattcctgaagatcatgttcagctacaacaacaaagagctgatcatcaacgagacagtgcccaacagattcagccctaagagccccgataaggcccacctgaacctgcacatcaacagcctggaactgggcgacagcgccgtgtacttttgtgccagcagccagttctgggatggcgctggcgacgagcagtattttggccctggcaccagactgaccgtgaccgaggacctgaacaaggtgttccctccggaggtggccgtgttcgagcccagcaaagccgagatcgcgcacacccagaaggccaccctggtgtgcctggccaccggcttcttccccgaccacgtggagctgagctggtgggtgaacggcaaggaggtgcacagcggcgtgagcaccgacccccagcccctgaaggagcagcccgccctgaacgacagccgctactgcctgagcagccgcctgcgcgtgagcgccaccttctggcagaacccccgcaaccacttccgctgccaggtgcagttctacggcctgagcgagaacgacgagtggacccaggaccgcgccaagcccgtgacccagatcgtgagcgccgaggcctggggccgcgccgactgcggcattaccagcgcgagctaccatcagggcgtgctgagcgccaccatcctgtacgagatcctgctgggcaaggccaccctgtacgccgtgctggtgagcgccctggtgctgatggcgatggtgaagcgcaaggacttctga

SEQ ID NO: 56 - protein, 10 aa, Homo sapiens
KLYGLDWAEL

SEQ ID NO: 57 - protein, 272 aa, Artificial Sequence
  murinized
MSLSSLLKVVTASLWLGPGIAQKITQTQPGMFVQEKEAVTLDCTYDTSDQSYGLFWYKQPSSGEMIFLIYQGSYDEQNATEGRYSLNFQKARKSANLVISASQLGDSAMYFCAMSGDSAGNMLTFGGGTRLMVKPHIQNPEPAVYQLKDPRSQDSTLCLFTDFDSQINVPKTMESGTFITDKTVLDMKAMDSKSNGAIAWSNQTSFTCQDIFKETNATYPSSDVPCDATLTEKSFETDMNLNFQNLSVMGLRILLLKVAGFNLLMTLRLWSS

SEQ ID NO: 58 - protein, 308 aa, Artificial Sequence
  murinized
MASLLFFCGAFYLLGTGSMDADVTQTPRNRITKTGKRIMLECSQTKGHDRMYWYRQDPGLGLRLIYYSFDVKDINKGEISDGYSVSRQAQAKFSLSLESAIPNQTALYFCATSDWDRSGDKETQYFGPGTRLLVLEDLRNVTPPKVTLFEPSKAEIANKQKATLVCLARGFFPDHVELSWWVNGKEVHSGVSTDPQAYKESNYSYCLSSRLRVSATFWHNPRNHFRCQVQFHGLSEEDKWPEGSPKPVTQNISAEAWGRADCGITSASYHQGVLSATILYEILLGKATLYAVLVSGLVLMAMVKKKNS

SEQ ID NO: 59 - protein, 273 aa, Artificial Sequence
  murinized
MSLSSLLKVVTASLWLGPGIAQKITQTQPGMFVQEKEAVTLDCTYDTSDPSYGLFWYKQPSSGEMIFLIYQGSYDQQNATEGRYSLNFQKARKSANLVISASQLGDSAMYFCAMSGGYTGGFKTIFGAGTRLFVKANIQNPEPAVYQLKDPRSQDSTLCLFTDFDSQINVPKTMESGTFITDKTVLDMKAMDSKSNGAIAWSNQTSFTCQDIFKETNATYPSSDVPCDATLTEKSFETDMNLNFQNLSVMGLRILLLKVAGFNLLMTLRLWSS

SEQ ID NO: 60 - protein, 304 aa, Artificial Sequence
  murinized
MGFRLLCCVAFCLLGAGPVDSGVTQTPKHLITATGQRVTLRCSPRSGDLSVYWYQQSLDQGLQFLIQYYNGEERAKGNILERFSAQQFPDLHSELNLSSLELGDSALYFCASSGGDGDEQFFGPGTRLTVLEDLRNVTPPKVTLFEPSKAEIANKQKATLVCLARGFFPDHVELSWWVNGKEVHSGVSTDPQAYKESNYSYCLSSRLRVSATFWHNPRNHFRCQVQFHGLSEEDKWPEGSPKPVTQNISAEAWGRADCGITSASYHQGVLSATILYEILLGKATLYAVLVSGLVLMAMVKKKNS

SEQ ID NO: 61 - protein, 269 aa, Artificial Sequence
  murinized
MTSIRAVFIFLWLQLDLVNGENVEQHPSTLSVQEGDSAVIKCTYSDSASNYFPWYKQELGKRPQLIIDIRSNVGEKKDQRIAVTLNKTAKHFSLHITETQPEDSAVYFCAASRGTGFQKLVFGTGTRLLVSPNIQNPEPAVYQLKDPRSQDSTLCLFTDFDSQINVPKTMESGTFITDKTVLDMKAMDSKSNGAIAWSNQTSFTCQDIFKETNATYPSSDVPCDATLTEKSFETDMNLNFQNLSVMGLRILLLKVAGFNLLMTLRLWSS

SEQ ID NO: 62 - protein, 307 aa, Artificial Sequence
  murinized
MGCRLLCCVVFCLLQAGPLDTAVSQTPKYLVTQMGNDKSIKCEQNLGHDTMYWYKQDSKKFLKIMFSYNNKELIINETVPNRFSPKSPDKAHLNLHINSLELGDSAVYFCASSQFWDGAGDEQYFGPGTRLTVTEDLRNVTPPKVTLFEPSKAEIANKQKATLVCLARGFFPDHVELSWWVNGKEVHSGVSTDPQAYKESNYSYCLSSRLRVSATFWHNPRNHFRCQVQFHGLSEEDKWPEGSPKPVTQNISAEAWGRADCGITSASYHQGVLSATILYEILLGKATLYAVLVSGLVLMAMVKKKNS

SEQ ID NO: 63 - DNA, 21 bp, Artificial Sequence
  human optimized
acttcagaccagtcgtacggt

SEQ ID NO: 64 - DNA, 24 bp, Artificial Sequence
  human optimized
cagggatcgtacgacgagcagaac

SEQ ID NO: 65 - DNA, 42 bp, Artificial Sequence
  human optimized
tgcgcaatgtccggcgatagcgcaggaaacatgctgactttc

SEQ ID NO: 66 - DNA, 15 bp, Artificial Sequence
  human optimized
aagggccacgaccgc

SEQ ID NO: 67 - DNA, 18 bp, Artificial Sequence
  human optimized
tccttcgacgtgaaggac

SEQ ID NO: 68 - DNA, 51 bp, Artificial Sequence
  human optimized
tgtgccacctcggattgggaccgatccggcgacaaggaaactcagtacttc

SEQ ID NO: 69 - DNA, 831 bp, human optimized
atgagcctctcttccctgctcaaagtggtcactgcctccctgtggctgggaccgggaatcgcccagaagatcactcagacccagcctggaatgttcgtgcaagagaaagaggccgtgaccctggattgtacttatgacacttcagaccagtcgtacggtttgttctggtacaagcagccgtcctccggagaaatgatcttcctgatctaccagggatcgtacgacgagcagaacgctaccgagggcagatattccctcaacttccaaaaggcccggaaatccgcgaacctcgtgatctcggcctcacaacttggggactccgctatgtatttctgcgcaatgtccggcgatagcgcaggaaacatgctgactttcggcggtggaactaggctgatggtcaagccccacattcaaaaccctgacccagcagtctaccagttgcgggattccaagtcttccgataaatccgtgtgtctctttacagacttcgatagccagaccaacgtgtcccagagcaaagacagcgacgtgtacattactgacaagactgtgctggacatgcggtccatggacttcaagagcaactccgccgtcgcttggtccaacaagtctgactttgcgtgcgcgaacgctttcaacaacagcattatcccggaggacacctttttcccttcccccgagtcaagctgcgatgtcaagcttgtggaaaagtcgttcgaaaccgacaccaacctgaacttccagaacctgtccgtcatcgggttccgcattctgctgctgaaggtcgccggcttcaatctcctgatgactctccgcttgtggtcctcataa

SEQ ID NO: 70 - DNA, 936 bp, human optimized
atggcgtccctgctgttcttctgcggtgccttctaccttctgggaaccggctcgatggacgccgacgtgacccaaacccctcgcaaccgcatcaccaagactggaaagcggatcatgctggaatgctcccagaccaagggccacgaccgcatgtactggtacagacaggacccgggtctgggattgcgcctgatctactactccttcgacgtgaaggacatcaacaagggggagatctccgatggatactcagtctcgagacaagcccaggctaagttttccctgtccctcgaatccgccattcccaatcagaccgcgctgtacttctgtgccacctcggattgggaccgatccggcgacaaggaaactcagtacttcggaccaggaaccaggctcctggtgctggaggatctgaacaaggtgttcccgccggaagtggcagtgttcgagccatccgaagccgagatctcgcatacgcagaaggccaccctcgtgtgcctggccactgggtttttccctgaccacgtggagctctcgtggtgggtcaacggaaaggaagtgcacagcggtgtctcaaccgacccgcaacctctcaaggaacagcccgcgctcaatgattcgcggtactgcctgagcagccggctcagagtgtccgccactttctggcaaaacccgcggaaccatttccggtgccaagtgcaattctacgggctgtcggaaaacgacgaatggacccaggacagggccaagcccgtgacccagattgtgtccgctgaagcctgggggagagctgattgcggtttcaccagcgtgtcgtatcagcagggcgtgctgtcagccaccattctgtacgaaatcctcctggggaaggccacactgtacgccgtgctcgtgtccgccctggtgctgatggccatggtcaagcggaaggacttc

SEQ ID NO: 71 - DNA, 21 bp, human optimized
acctccgacccgtcctacggg

SEQ ID NO: 72 - DNA, 24 bp, human optimized
caaggctcctatgatcagcagaac

SEQ ID NO: 73 - DNA, 45 bp, Artificial Sequence
  human optimized
tgtgccatgtcgggcggatacaccgggggattcaagaccattttc

SEQ ID NO: 74 - DNA, 15 bp, Artificial Sequence
  human optimized
tctggcgacctctcc

SEQ ID NO: 75 - DNA, 18 bp, Artificial Sequence
  human optimized
tactacaacggagaggag

SEQ ID NO: 76 - DNA, 39 bp, Artificial Sequence
  human optimized
tgcgcaagcagcggtggtgacggggatgaacagttcttt

SEQ ID NO: 77 - DNA, 834 bp, Artificial Sequence
  human optimized
atgtcccttagctcactgctgaaagtggtcactgcgagcctgtggctgggaccaggcattgctcaaaagatcacccagactcagcctgggatgttcgtgcaagagaaggaagccgtgaccctcgactgcacttacgacacctccgacccgtcctacgggctgttctggtacaagcagccgtcctccggagagatgatcttcctcatctaccaaggctcctatgatcagcagaacgccaccgaaggacgctacagcctgaacttccagaaggctcggaagtcggcgaacctcgtgatcagcgcatcccaactgggggacagcgccatgtacttctgtgccatgtcgggcggatacaccgggggattcaagaccattttcggggccggcactagactgttcgtgaaggccaacatccagaatcctgatccggcggtgtatcagctgcgcgactccaagtcttccgataaatccgtgtgtctctttacagacttcgactcccaaaccaacgtgtcacagtccaaggacagcgatgtgtacatcaccgacaaaaccgtgctggacatgcggtccatggacttcaagtcaaacagcgcagtcgcctggtccaacaagtccgacttcgcctgtgcgaacgccttcaacaactccatcattccggaagatacctttttcccttcacctgagtcgagctgtgatgtgaagctcgtggaaaagtcgtttgaaacggacaccaacctgaactttcagaacctgtccgtgattggtttccgcatcctgctgctgaaggtcgccggcttcaacttgctgatgacgctccggctgtggtcctcgtaa

SEQ ID NO: 78 - DNA, 930 bp, Artificial Sequence
  human optimized
atgggattccgccttctgtgctgcgtggccttctgcttgcttggagctggtcccgtcgactcgggagtgacccagacgccgaagcacttgattaccgctactgggcagcgcgtgactctgcgatgctcaccacggtctggcgacctctccgtgtactggtatcagcagagcctggaccagggactgcagttcctgatccagtactacaacggagaggagcgggctaagggaaacatactggagcggttctcggcgcaacaattccccgatctgcactccgaactgaacctgtcctccctggaattgggagactccgccctgtacttctgcgcaagcagcggtggtgacggggatgaacagttctttggccctggaaccagactcaccgtgctcgaggacctcaagaacgtgttcccacccgaagtcgcggtgttcgagccctccgaagcggaaatcagccatactcagaaagccactctcgtgtgcctggccaccggattctacccggaccacgtcgagctctcttggtgggtgaacgggaaagaggtccacagcggcgtgagcactgatccgcagccgctgaaggaacaacccgccttgaacgactcgcggtactgtctgtcctcccggctgagagtgtcggccaccttctggcaaaaccccaggaaccactttaggtgccaagtccagttctacggcctgagcgaaaacgatgagtggacccaggacagagccaagcctgtgacccagattgtgtcagccgaggcttggggtagagcagactgcggattcacctccgagtcctaccaacaaggcgtcctctcggcgaccattctgtacgaaatcctgcttgggaaggccactctgtacgccgtgctggtgtccgccctggtgctgatggccatggtcaagcggaaggactcccggggg

SEQ ID NO: 79 - DNA, 18 bp, Artificial Sequence
  human optimized
gactcagcatcaaactat

SEQ ID NO: 80 - DNA, 21 bp, Artificial Sequence
  human optimized
atccgctccaacgtcggagag

SEQ ID NO: 81 - DNA, 42 bp, Artificial Sequence
  human optimized
tgtgcggcctcgaggggcactgggtttcagaagctcgtgttc

SEQ ID NO: 82 - DNA, 15 bp, Artificial Sequence
  human optimized
ctcggacacgacacc

SEQ ID NO: 83 - DNA, 18 bp, Artificial Sequence
  human optimized
tacaacaacaaggaactg

SEQ ID NO: 84 - DNA, 48 bp, Artificial Sequence
  human optimized
tgcgcgtccagccagttctgggacggagcgggcgacgaacagtacttc

SEQ ID NO: 85 - DNA, 819 bp, Artificial Sequence
  human optimized
atgacgtccattagagccgtgttcattttcctgtggctgcaactggacctcgtgaatggagaaaacgtcgagcagcacccatccaccctgagcgtgcaggagggagactccgcagtcatcaagtgcacttactccgactcagcatcaaactatttcccgtggtataagcaggaactcggaaagcggcctcagctcatcattgacatccgctccaacgtcggagagaagaaggaccagagaattgccgtgacactcaacaagaccgccaagcatttctcccttcacatcaccgaaacccagcccgaggacagcgccgtctacttttgtgcggcctcgaggggcactgggtttcagaagctcgtgttcggcactgggacccggctgctggtgtcgccaaacatccagaatccagaccccgcggtgtaccagctgagagactcgaagtcttccgataaatccgtgtgtctctttacagacttcgatagccagactaacgtgtcccagtccaaggactccgatgtgtacatcaccgacaagactgtgctggatatgcggagcatggactttaagtccaattcagcggtcgcgtggagcaacaagtccgacttcgcctgcgctaacgctttcaacaactccattatcccggaggataccttcttcccgtcaccggaatcctcgtgcgacgtgaagctggtcgagaagtccttcgaaaccgataccaacctgaacttccaaaacctctccgtgatcggcttcagaatcctgctgctgaaagtggctggcttcaatttgctgatgaccctgcggctctggagcagc

SEQ ID NO: 86 - DNA, 930 bp, Artificial Sequence
  human optimized
atgggttgtcggttgctgtgttgcgtcgtgttctgccttcttcaagctggtcctctcgatactgccgtgagccaaacccctaagtaccttgtcacccaaatgggcaacgacaagtccatcaaatgcgaacagaacctcggacacgacaccatgtactggtacaaacaggattccaagaagttcctgaagattatgttctcatacaacaacaaggaactgattatcaacgaaactgtgccgaaccggttctcaccgaagtcgcctgacaaggctcatctcaacttgcatatcaactcgctggagctcggcgactccgccgtgtacttctgcgcgtccagccagttctgggacggagcgggcgacgaacagtacttcggcccgggcactcggctgaccgtgaccgaagatctgaacaaagtgttcccccccgaagtggccgtgttcgaaccttccgaggccgagatcagccacacccaaaaggccactctggtctgcctggccaccggtttcttccccgatcacgtggaactgtcttggtgggtgaacggaaaagaagtgcactcgggggtgtccacggacccccagcctctgaaggaacagccggcactgaatgactcacgctactgtctgtcgtcacggctgcgcgtgtcggccaccttctggcaaaacccgcgaaaccactttcgctgccaagtgcagttttacgggctttccgagaacgacgagtggactcaggacagagcgaagcccgtgacccaaatcgtgtccgccgaggcctggggacgcgccgactgcggtttcacctccgtgagctaccaacagggcgtgctgtcagctaccatcctttacgagatcctcctgggaaaggccaccctctacgccgtcctggtgtccgcactggtgctgatggctatggtcaagcggaaggat

SEQ ID NO: 87 - protein, 276 aa, Homo sapiens
MSLSSLLKVVTASLWLGPGIAQKITQTQPGMFVQEKEAVTLDCTYDTSDQSYGLFWYKQPSSGEMIFLIYQGSYDEQNATEGRYSLNFQKARKSANLVISASQLGDSAMYFCAMSGDSAGNMLTFGGGTRLMVKPHIQNPDPAVYQLRDSKSSDKSVCLFTDFDSQTNVSQSKDSDVYITDKTVLDMRSMDFKSNSAVAWSNKSDFACANAFNNSIIPEDTFFPSPESSCDVKLVEKSFETDTNLNFQNLSVIGFRILLLKVAGFNLLMTLRLWSS

SEQ ID NO: 88 - protein, 312 aa, Homo sapiens
MASLLFFCGAFYLLGTGSMDADVTQTPRNRITKTGKRIMLECSQTKGHDRMYWYRQDPGLGLRLIYYSFDVKDINKGEISDGYSVSRQAQAKFSLSLESAIPNQTALYFCATSDWDRSGDKETQYFGPGTRLLVLEDLNKVFPPEVAVFEPSEAEISHTQKATLVCLATGFFPDHVELSWWVNGKEVHSGVSTDPQPLKEQPALNDSRYCLSSRLRVSATFWQNPRNHFRCQVQFYGLSENDEWTQDRAKPVTQIVSAEAWGRADCGFTSVSYQQGVLSATILYEILLGKATLYAVLVSALVLMAMVKRKDF

SEQ ID NO: 89 - protein, 277 aa, Homo sapiens
MSLSSLLKVVTASLWLGPGIAQKITQTQPGMFVQEKEAVTLDCTYDTSDPSYGLFWYKQPSSGEMIFLIYQGSYDQQNATEGRYSLNFQKARKSANLVISASQLGDSAMYFCAMSGGYTGGFKTIFGAGTRLFVKANIQNPDPAVYQLRDSKSSDKSVCLFTDFDSQTNVSQSKDSDVYITDKTVLDMRSMDFKSNSAVAWSNKSDFACANAFNNSIIPEDTFFPSPESSCDVKLVEKSFETDTNLNFQNLSVIGFRILLLKVAGFNLLMTLRLWSS

SEQ ID NO: 90 - protein, 310 aa, Homo sapiens
MGFRLLCCVAFCLLGAGPVDSGVTQTPKHLITATGQRVTLRCSPRSGDLSVYWYQQSLDQGLQFLIQYYNGEERAKGNILERFSAQQFPDLHSELNLSSLELGDSALYFCASSGGDGDEQFFGPGTRLTVLEDLKNVFPPEVAVFEPSEAEISHTQKATLVCLATGFYPDHVELSWWVNGKEVHSGVSTDPQPLKEQPALNDSRYCLSSRLRVSATFWQNPRNHFRCQVQFYGLSENDEWTQDRAKPVTQIVSAEAWGRADCGFTSESYQQGVLSATILYEILLGKATLYAVLVSALVLMAMVKRKDSRG

SEQ ID NO: 91 - protein, 273 aa, Homo sapiens
MTSIRAVFIFLWLQLDLVNGENVEQHPSTLSVQEGDSAVIKCTYSDSASNYFPWYKQELGKRPQLIIDIRSNVGEKKDQRIAVTLNKTAKHFSLHITETQPEDSAVYFCAASRGTGFQKLVFGTGTRLLVSPNIQNPDPAVYQLRDSKSSDKSVCLFTDFDSQTNVSQSKDSDVYITDKTVLDMRSMDFKSNSAVAWSNKSDFACANAFNNSIIPEDTFFPSPESSCDVKLVEKSFETDTNLNFQNLSVIGFRILLLKVAGFNLLMTLRLWSS

SEQ ID NO: 92 - protein, 310 aa, Homo sapiens
MGCRLLCCVVFCLLQAGPLDTAVSQTPKYLVTQMGNDKSIKCEQNLGHDTMYWYKQDSKKFLKIMFSYNNKELIINETVPNRFSPKSPDKAHLNLHINSLELGDSAVYFCASSQFWDGAGDEQYFGPGTRLTVTEDLNKVFPPEVAVFEPSEAEISHTQKATLVCLATGFFPDHVELSWWVNGKEVHSGVSTDPQPLKEQPALNDSRYCLSSRLRVSATFWQNPRNHFRCQVQFYGLSENDEWTQDRAKPVTQIVSAEAWGRADCGFTSVSYQQGVLSATILYEILLGKATLYAVLVSALVLMAMVKRKD

SEQ ID NO: 93 - DNA, 1833 bp, Artificial Sequence
  human optimized
atggcgtccctgctgttcttctgcggtgccttctaccttctgggaaccggctcgatggacgccgacgtgacccaaacccctcgcaaccgcatcaccaagactggaaagcggatcatgctggaatgctcccagaccaagggccacgaccgcatgtactggtacagacaggacccgggtctgggattgcgcctgatctactactccttcgacgtgaaggacatcaacaagggggagatctccgatggatactcagtctcgagacaagcccaggctaagttttccctgtccctcgaatccgccattcccaatcagaccgcgctgtacttctgtgccacctcggattgggaccgatccggcgacaaggaaactcagtacttcggaccaggaaccaggctcctggtgctggaggatctgaacaaggtgttcccgccggaagtggcagtgttcgagccatccgaagccgagatctcgcatacgcagaaggccaccctcgtgtgcctggccactgggtttttccctgaccacgtggagctctcgtggtgggtcaacggaaaggaagtgcacagcggtgtctcaaccgacccgcaacctctcaaggaacagcccgcgctcaatgattcgcggtactgcctgagcagccggctcagagtgtccgccactttctggcaaaacccgcggaaccatttccggtgccaagtgcaattctacgggctgtcggaaaacgacgaatggacccaggacagggccaagcccgtgacccagattgtgtccgctgaagcctgggggagagctgattgcggtttcaccagcgtgtcgtatcagcagggcgtgctgtcagccaccattctgtacgaaatcctcctggggaaggccacactgtacgccgtgctcgtgtccgccctggtgctgatggccatggtcaagcggaaggacttcggcagcggagctaccaacttctccctgctgaagcaggccggcgatgtggaagaaaatcccggacctatgagcctctcttccctgctcaaagtggtcactgcctccctgtggctgggaccgggaatcgcccagaagatcactcagacccagcctggaatgttcgtgcaagagaaagaggccgtgaccctggattgtacttatgacacttcagaccagtcgtacggtttgttctggtacaagcagccgtcctccggagaaatgatcttcctgatctaccagggatcgtacgacgagcagaacgctaccgagggcagatattccctcaacttccaaaaggcccggaaatccgcgaacctcgtgatctcggcctcacaacttggggactccgctatgtatttctgcgcaatgtccggcgatagcgcaggaaacatgctgactttcggcggtggaactaggctgatggtcaagccccacattcaaaaccctgacccagcagtctaccagttgcgggattccaagtcttccgataaatccgtgtgtctctttacagacttcgatagccagaccaacgtgtcccagagcaaagacagcgacgtgtacattactgacaagactgtgctggacatgcggtccatggacttcaagagcaactccgccgtcgcttggtccaacaagtctgactttgcgtgcgcgaacgctttcaacaacagcattatcccggaggacacctttttcccttcccccgagtcaagctgcgatgtcaagcttgtggaaaagtcgttcgaaaccgacaccaacctgaacttccagaacctgtccgtcatcgggttccgcattctgctgctgaaggtcgccggcttcaatctcctgatgactctccgcttgtggtcctcataa

SEQ ID NO: 94 - protein, 610 aa, Artificial Sequence
  human optimized
MASLLFFCGAFYLLGTGSMDADVTQTPRNRITKTGKRIMLECSQTKGHDRMYWYRQDPGLGLRLIYYSFDVKDINKGEISDGYSVSRQAQAKFSLSLESAIPNQTALYFCATSDWDRSGDKETQYFGPGTRLLVLEDLNKVFPPEVAVFEPSEAEISHTQKATLVCLATGFFPDHVELSWWVNGKEVHSGVSTDPQPLKEQPALNDSRYCLSSRLRVSATFWQNPRNHFRCQVQFYGLSENDEWTQDRAKPVTQIVSAEAWGRADCGFTSVSYQQGVLSATILYEILLGKATLYAVLVSALVLMAMVKRKDFGSGATNFSLLKQAGDVEENPGPMSLSSLLKVVTASLWLGPGIAQKITQTQPGMFVQEKEAVTLDCTYDTSDQSYGLFWYKQPSSGEMIFLIYQGSYDEQNATEGRYSLNFQKARKSANLVISASQLGDSAMYFCAMSGDSAGNMLTFGGGTRLMVKPHIQNPDPAVYQLRDSKSSDKSVCLFTDFDSQTNVSQSKDSDVYITDKTVLDMRSMDFKSNSAVAWSNKSDFACANAFNNSIIPEDTFFPSPESSCDVKLVEKSFETDTNLNFQNLSVIGFRILLLKVAGFNLLMTLRLWSS

SEQ ID NO: 95 - DNA, 1842 bp, Artificial Sequence
  human optimized
atgggattccgccttctgtgctgcgtggccttctgcttgcttggagctggtcccgtcgactcgggagtgacccagacgccgaagcacttgattaccgctactgggcagcgcgtgactctgcgatgctcaccacggtctggcgacctctccgtgtactggtatcagcagagcctggaccagggactgcagttcctgatccagtactacaacggagaggagcgggctaagggaaacatactggagcggttctcggcgcaacaattccccgatctgcactccgaactgaacctgtcctccctggaattgggagactccgccctgtacttctgcgcaagcagcggtggtgacggggatgaacagttctttggccctggaaccagactcaccgtgctcgaggacctcaagaacgtgttcccacccgaagtcgcggtgttcgagccctccgaagcggaaatcagccatactcagaaagccactctcgtgtgcctggccaccggattctacccggaccacgtcgagctctcttggtgggtgaacgggaaagaggtccacagcggcgtgagcactgatccgcagccgctgaaggaacaacccgccttgaacgactcgcggtactgtctgtcctcccggctgagagtgtcggccaccttctggcaaaaccccaggaaccactttaggtgccaagtccagttctacggcctgagcgaaaacgatgagtggacccaggacagagccaagcctgtgacccagattgtgtcagccgaggcttggggtagagcagactgcggattcacctccgagtcctaccaacaaggcgtcctctcggcgaccattctgtacgaaatcctgcttgggaaggccactctgtacgccgtgctggtgtccgccctggtgctgatggccatggtcaagcggaaggactcccgggggagagcaaagaggggatcgggagccaccaattttagcctgctgaagcaggccggcgatgtggaagaaaatcctggccccatgtcccttagctcactgctgaaagtggtcactgcgagcctgtggctgggaccaggcattgctcaaaagatcacccagactcagcctgggatgttcgtgcaagagaaggaagccgtgaccctcgactgcacttacgacacctccgacccgtcctacgggctgttctggtacaagcagccgtcctccggagagatgatcttcctcatctaccaaggctcctatgatcagcagaacgccaccgaaggacgctacagcctgaacttccagaaggctcggaagtcggcgaacctcgtgatcagcgcatcccaactgggggacagcgccatgtacttctgtgccatgtcgggcggatacaccgggggattcaagaccattttcggggccggcactagactgttcgtgaaggccaacatccagaatcctgatccggcggtgtatcagctgcgcgactccaagtcttccgataaatccgtgtgtctctttacagacttcgactcccaaaccaacgtgtcacagtccaaggacagcgatgtgtacatcaccgacaaaaccgtgctggacatgcggtccatggacttcaagtcaaacagcgcagtcgcctggtccaacaagtccgacttcgcctgtgcgaacgccttcaacaactccatcattccggaagatacctttttcccttcacctgagtcgagctgtgatgtgaagctcgtggaaaagtcgtttgaaacggacaccaacctgaactttcagaacctgtccgtgattggtttccgcatcctgctgctgaaggtcgccggcttcaacttgctgatgacgctccggctgtggtcctcgtaa

SEQ ID NO: 96 - protein, 613 aa, Artificial Sequence
  human optimized
MGFRLLCCVAFCLLGAGPVDSGVTQTPKHLITATGQRVTLRCSPRSGDLSVYWYQQSLDQGLQFLIQYYNGEERAKGNILERFSAQQFPDLHSELNLSSLELGDSALYFCASSGGDGDEQFFGPGTRLTVLEDLKNVFPPEVAVFEPSEAEISHTQKATLVCLATGFYPDHVELSWWVNGKEVHSGVSTDPQPLKEQPALNDSRYCLSSRLRVSATFWQNPRNHFRCQVQFYGLSENDEWTQDRAKPVTQIVSAEAWGRADCGFTSESYQQGVLSATILYEILLGKATLYAVLVSALVLMAMVKRKDSRGRAKRGSGATNFSLLKQAGDVEENPGPMSLSSLLKVVTASLWLGPGIAQKITQTQPGMFVQEKEAVTLDCTYDTSDPSYGLFWYKQPSSGEMIFLIYQGSYDQQNATEGRYSLNFQKARKSANLVISASQLGDSAMYFCAMSGGYTGGFKTIFGAGTRLFVKANIQNPDPAVYQLRDSKSSDKSVCLFTDFDSQTNVSQSKDSDVYITDKTVLDMRSMDFKSNSAVAWSNKSDFACANAFNNSIIPEDTFFPSPESSCDVKLVEKSFETDTNLNFQNLSVIGFRILLLKVAGFNLLMTLRLWSS

SEQ ID NO: 97 - DNA, 1830 bp, Artificial Sequence
  human optimized
atgggttgtcggttgctgtgttgcgtcgtgttctgccttcttcaagctggtcctctcgatactgccgtgagccaaacccctaagtaccttgtcacccaaatgggcaacgacaagtccatcaaatgcgaacagaacctcggacacgacaccatgtactggtacaaacaggattccaagaagttcctgaagattatgttctcatacaacaacaaggaactgattatcaacgaaactgtgccgaaccggttctcaccgaagtcgcctgacaaggctcatctcaacttgcatatcaactcgctggagctcggcgactccgccgtgtacttctgcgcgtccagccagttctgggacggagcgggcgacgaacagtacttcggcccgggcactcggctgaccgtgaccgaagatctgaacaaagtgttcccccccgaagtggccgtgttcgaaccttccgaggccgagatcagccacacccaaaaggccactctggtctgcctggccaccggtttcttccccgatcacgtggaactgtcttggtgggtgaacggaaaagaagtgcactcgggggtgtccacggacccccagcctctgaaggaacagccggcactgaatgactcacgctactgtctgtcgtcacggctgcgcgtgtcggccaccttctggcaaaacccgcgaaaccactttcgctgccaagtgcagttttacgggctttccgagaacgacgagtggactcaggacagagcgaagcccgtgacccaaatcgtgtccgccgaggcctggggacgcgccgactgcggtttcacctccgtgagctaccaacagggcgtgctgtcagctaccatcctttacgagatcctcctgggaaaggccaccctctacgccgtcctggtgtccgcactggtgctgatggctatggtcaagcggaaggattttagggccaaacgcgggtccggagcgaccaacttctcgctgttgaagcaggccggcgatgtggaagagaaccctggaccgatgacgtccattagagccgtgttcattttcctgtggctgcaactggacctcgtgaatggagaaaacgtcgagcagcacccatccaccctgagcgtgcaggagggagactccgcagtcatcaagtgcacttactccgactcagcatcaaactatttcccgtggtataagcaggaactcggaaagcggcctcagctcatcattgacatccgctccaacgtcggagagaagaaggaccagagaattgccgtgacactcaacaagaccgccaagcatttctcccttcacatcaccgaaacccagcccgaggacagcgccgtctacttttgtgcggcctcgaggggcactgggtttcagaagctcgtgttcggcactgggacccggctgctggtgtcgccaaacatccagaatccagaccccgcggtgtaccagctgagagactcgaagtcttccgataaatccgtgtgtctctttacagacttcgatagccagactaacgtgtcccagtccaaggactccgatgtgtacatcaccgacaagactgtgctggatatgcggagcatggactttaagtccaattcagcggtcgcgtggagcaacaagtccgacttcgcctgcgctaacgctttcaacaactccattatcccggaggataccttcttcccgtcaccggaatcctcgtgcgacgtgaagctggtcgagaagtccttcgaaaccgataccaacctgaacttccaaaacctctccgtgatcggcttcagaatcctgctgctgaaagtggctggcttcaatttgctgatgaccctgcggctctggagcagc

SEQ ID NO: 98 - protein, 610 aa, Artificial Sequence
  human optimized
MGCRLLCCVVFCLLQAGPLDTAVSQTPKYLVTQMGNDKSIKCEQNLGHDTMYWYKQDSKKFLKIMFSYNNKELIINETVPNRFSPKSPDKAHLNLHINSLELGDSAVYFCASSQFWDGAGDEQYFGPGTRLTVTEDLNKVFPPEVAVFEPSEAEISHTQKATLVCLATGFFPDHVELSWWVNGKEVHSGVSTDPQPLKEQPALNDSRYCLSSRLRVSATFWQNPRNHFRCQVQFYGLSENDEWTQDRAKPVTQIVSAEAWGRADCGFTSVSYQQGVLSATILYEILLGKATLYAVLVSALVLMAMVKRKDFRAKRGSGATNFSLLKQAGDVEENPGPMTSIRAVFIFLWLQLDLVNGENVEQHPSTLSVQEGDSAVIKCTYSDSASNYFPWYKQELGKRPQLIIDIRSNVGEKKDQRIAVTLNKTAKHFSLHITETQPEDSAVYFCAASRGTGFQKLVFGTGTRLLVSPNIQNPDPAVYQLRDSKSSDKSVCLFTDFDSQTNVSQSKDSDVYITDKTVLDMRSMDFKSNSAVAWSNKSDFACANAFNNSIIPEDTFFPSPESSCDVKLVEKSFETDTNLNFQNLSVIGFRILLLKVAGFNLLMTLRLWSS

SEQ ID NO: 99 - DNA, 828 bp, Artificial Sequence
  TCR-7 a complete
atgagcctctcttccctgctcaaagtggtcactgcctccctgtggctgggaccgggaatcgcccagaagatcactcagacccagcctggaatgttcgtgcaagagaaagaggccgtgaccctggattgtacttatgacacttcagaccagtcgtacggtttgttctggtacaagcagccgtcctccggagaaatgatcttcctgatctaccagggatcgtacgacgagcagaacgctaccgagggcagatattccctcaacttccaaaaggcccggaaatccgcgaacctcgtgatctcggcctcacaacttggggactccgctatgtatttctgcgcaatgtccggcgatagcgcaggaaacatgctgactttcggcggtggaactaggctgatggtcaagccccacattcaaaaccctgacccagcagtctaccagttgcgggattccaagtcttccgataaatccgtgtgtctctttacagacttcgatagccagaccaacgtgtcccagagcaaagacagcgacgtgtacattactgacaagactgtgctggacatgcggtccatggacttcaagagcaactccgccgtcgcttggtccaacaagtctgactttgcgtgcgcgaacgctttcaacaacagcattatcccggaggacacctttttcccttccagcgacgtcccctgcgatgtcaagcttgtggaaaagtcgttcgaaaccgacaccaacctgaacttccagaacctgctagtgattgtgctccgcattctgctgctgaaggtcgccggcttcaatctcctgatgactctccgcttgtggtcctca

SEQ ID NO: 100 - DNA, 936 bp, Artificial Sequence
  TCR-7 b complete
atggcgtccctgctgttcttctgcggtgccttctaccttctgggaaccggctcgatggacgccgacgtgacccaaacccctcgcaaccgcatcaccaagactggaaagcggatcatgctggaatgctcccagaccaagggccacgaccgcatgtactggtacagacaggacccgggtctgggattgcgcctgatctactactccttcgacgtgaaggacatcaacaagggggagatctccgatggatactcagtctcgagacaagcccaggctaagttttccctgtccctcgaatccgccattcccaatcagaccgcgctgtacttctgtgccacctcggattgggaccgatccggcgacaaggaaactcagtacttcggaccaggaaccaggctcctggtgctggaggatctgaacaaggtgttcccgccggaagtggcagtgttcgagccatccaaggcggagatcgcccatacgcagaaggccaccctcgtgtgcctggccactgggtttttccctgaccacgtggagctctcgtggtgggtcaacggaaaggaagtgcacagcggtgtctcaaccgacccgcaacctctcaaggaacagcccgcgctcaatgattcgcggtactgcctgagcagccggctcagagtgtccgccactttctggcaaaacccgcggaaccatttccggtgccaagtgcaattctacgggctgtcggaaaacgacgaatggacccaggacagggccaagcccgtgacccagattgtgtccgctgaagcctgggggagagctgattgcggtatcaccagcgccagctaccaccagggcgtgctgtcagccaccattctgtacgaaatcctcctggggaaggccacactgtacgccgtgctcgtgtccgccctggtgctgatggccatggtcaagcggaaggacttc

SEQ ID NO: 101 - DNA, 1833 bp, Artificial Sequence
  TCR-7 polycistronic construct
atggcgtccctgctgttcttctgcggtgccttctaccttctgggaaccggctcgatggacgccgacgtgacccaaacccctcgcaaccgcatcaccaagactggaaagcggatcatgctggaatgctcccagaccaagggccacgaccgcatgtactggtacagacaggacccgggtctgggattgcgcctgatctactactccttcgacgtgaaggacatcaacaagggggagatctccgatggatactcagtctcgagacaagcccaggctaagttttccctgtccctcgaatccgccattcccaatcagaccgcgctgtacttctgtgccacctcggattgggaccgatccggcgacaaggaaactcagtacttcggaccaggaaccaggctcctggtgctggaggatctgaacaaggtgttcccgccggaagtggcagtgttcgagccatccaaggcggagatcgcccatacgcagaaggccaccctcgtgtgcctggccactgggtttttccctgaccacgtggagctctcgtggtgggtcaacggaaaggaagtgcacagcggtgtctcaaccgacccgcaacctctcaaggaacagcccgcgctcaatgattcgcggtactgcctgagcagccggctcagagtgtccgccactttctggcaaaacccgcggaaccatttccggtgccaagtgcaattctacgggctgtcggaaaacgacgaatggacccaggacagggccaagcccgtgacccagattgtgtccgctgaagcctgggggagagctgattgcggtatcaccagcgccagctaccaccagggcgtgctgtcagccaccattctgtacgaaatcctcctggggaaggccacactgtacgccgtgctcgtgtccgccctggtgctgatggccatggtcaagcggaaggacttcggcagcggagctaccaacttctccctgctgaagcaggccggcgatgtggaagaaaatcccggacctatgagcctctcttccctgctcaaagtggtcactgcctccctgtggctgggaccgggaatcgcccagaagatcactcagacccagcctggaatgttcgtgcaagagaaagaggccgtgaccctggattgtacttatgacacttcagaccagtcgtacggtttgttctggtacaagcagccgtcctccggagaaatgatcttcctgatctaccagggatcgtacgacgagcagaacgctaccgagggcagatattccctcaacttccaaaaggcccggaaatccgcgaacctcgtgatctcggcctcacaacttggggactccgctatgtatttctgcgcaatgtccggcgatagcgcaggaaacatgctgactttcggcggtggaactaggctgatggtcaagccccacattcaaaaccctgacccagcagtctaccagttgcgggattccaagtcttccgataaatccgtgtgtctctttacagacttcgatagccagaccaacgtgtcccagagcaaagacagcgacgtgtacattactgacaagactgtgctggacatgcggtccatggacttcaagagcaactccgccgtcgcttggtccaacaagtctgactttgcgtgcgcgaacgctttcaacaacagcattatcccggaggacacctttttcccttccagcgacgtcccctgcgatgtcaagcttgtggaaaagtcgttcgaaaccgacaccaacctgaacttccagaacctgctagtgattgtgctccgcattctgctgctgaaggtcgccggcttcaatctcctgatgactctccgcttgtggtcctcataa

SEQ ID NO: 102 - protein, 276 aa, Artificial Sequence
  TCR-7 a complete
MSLSSLLKVVTASLWLGPGIAQKITQTQPGMFVQEKEAVTLDCTYDTSDQSYGLFWYKQPSSGEMIFLIYQGSYDEQNATEGRYSLNFQKARKSANLVISASQLGDSAMYFCAMSGDSAGNMLTFGGGTRLMVKPHIQNPDPAVYQLRDSKSSDKSVCLFTDFDSQTNVSQSKDSDVYITDKTVLDMRSMDFKSNSAVAWSNKSDFACANAFNNSIIPEDTFFPSSDVPCDVKLVEKSFETDTNLNFQNLLVIVLRILLLKVAGFNLLMTLRLWSS

SEQ ID NO: 103 - protein, 312 aa, Artificial Sequence; identical to SEQ ID NO: 11
  TCR-7 b complete

SEQ ID NO: 104 - protein, 610 aa, Artificial Sequence
  TCR-7 polyprotein
MASLLFFCGAFYLLGTGSMDADVTQTPRNRITKTGKRIMLECSQTKGHDRMYWYRQDPGLGLRLIYYSFDVKDINKGEISDGYSVSRQAQAKFSLSLESAIPNQTALYFCATSDWDRSGDKETQYFGPGTRLLVLEDLNKVFPPEVAVFEPSKAEIAHTQKATLVCLATGFFPDHVELSWWVNGKEVHSGVSTDPQPLKEQPALNDSRYCLSSRLRVSATFWQNPRNHFRCQVQFYGLSENDEWTQDRAKPVTQIVSAEAWGRADCGITSASYHQGVLSATILYEILLGKATLYAVLVSALVLMAMVKRKDFGSGATNFSLLKQAGDVEENPGPMSLSSLLKVVTASLWLGPGIAQKITQTQPGMFVQEKEAVTLDCTYDTSDQSYGLFWYKQPSSGEMIFLIYQGSYDEQNATEGRYSLNFQKARKSANLVISASQLGDSAMYFCAMSGDSAGNMLTFGGGTRLMVKPHIQNPDPAVYQLRDSKSSDKSVCLFTDFDSQTNVSQSKDSDVYITDKTVLDMRSMDFKSNSAVAWSNKSDFACANAFNNSIIPEDTFFPSSDVPCDVKLVEKSFETDTNLNFQNLLVIVLRILLLKVAGFNLLMTLRLWSS

SEQ ID NO: 105 - DNA, 831 bp, Artificial Sequence
  TCR-8 a complete
atgtcccttagctcactgctgaaagtggtcactgcgagcctgtggctgggaccaggcattgctcaaaagatcacccagactcagcctgggatgttcgtgcaagagaaggaagccgtgaccctcgactgcacttacgacacctccgacccgtcctacgggctgttctggtacaagcagccgtcctccggagagatgatcttcctcatctaccaaggctcctatgatcagcagaacgccaccgaaggacgctacagcctgaacttccagaaggctcggaagtcggcgaacctcgtgatcagcgcatcccaactgggggacagcgccatgtacttctgtgccatgtcgggcggatacaccgggggattcaagaccattttcggggccggcactagactgttcgtgaaggccaacatccagaatcctgatccggcggtgtatcagctgcgcgactccaagtcttccgataaatccgtgtgtctctttacagacttcgactcccaaaccaacgtgtcacagtccaaggacagcgatgtgtacatcaccgacaaaaccgtgctggacatgcggtccatggacttcaagtcaaacagcgcagtcgcctggtccaacaagtccgacttcgcctgtgcgaacgccttcaacaactccatcattccggaagatacctttttcccttcaagcgacgtcccctgtgatgtgaagctcgtggaaaagtcgtttgaaacggacaccaacctgaactttcagaacctgctagtgattgtgctccgcatcctgctgctgaaggtcgccggcttcaacttgctgatgacgctccggctgtggtcctcg

SEQ ID NO: 106 - DNA, 930 bp, Artificial Sequence
  TCR-8 b complete
atgggattccgccttctgtgctgcgtggccttctgcttgcttggagctggtcccgtcgactcgggagtgacccagacgccgaagcacttgattaccgctactgggcagcgcgtgactctgcgatgctcaccacggtctggcgacctctccgtgtactggtatcagcagagcctggaccagggactgcagttcctgatccagtactacaacggagaggagcgggctaagggaaacatactggagcggttctcggcgcaacaattccccgatctgcactccgaactgaacctgtcctccctggaattgggagactccgccctgtacttctgcgcaagcagcggtggtgacggggatgaacagttctttggccctggaaccagactcaccgtgctcgaggacctcaagaacgtgttcccacccgaagtcgcggtgttcgagccctccaaggcggagatcgcccatactcagaaagccactctcgtgtgcctggccaccggattctacccggaccacgtcgagctctcttggtgggtgaacgggaaagaggtccacagcggcgtgagcactgatccgcagccgctgaaggaacaacccgccttgaacgactcgcggtactgtctgtcctcccggctgagagtgtcggccaccttctggcaaaaccccaggaaccactttaggtgccaagtccagttctacggcctgagcgaaaacgatgagtggacccaggacagagccaagcctgtgacccagattgtgtcagccgaggcttggggtagagcagactgcggaatcaccagcgccagctaccaccaaggcgtcctctcggcgaccattctgtacgaaatcctgcttgggaaggccactctgtacgccgtgctggtgtccgccctggtgctgatggccatggtcaagcggaaggactcccggggg

SEQ ID NO: 107 - DNA, 1842 bp, Artificial Sequence
  TCR-8 polycistronic construct
atgggattccgccttctgtgctgcgtggccttctgcttgcttggagctggtcccgtcgactcgggagtgacccagacgccgaagcacttgattaccgctactgggcagcgcgtgactctgcgatgctcaccacggtctggcgacctctccgtgtactggtatcagcagagcctggaccagggactgcagttcctgatccagtactacaacggagaggagcgggctaagggaaacatactggagcggttctcggcgcaacaattccccgatctgcactccgaactgaacctgtcctccctggaattgggagactccgccctgtacttctgcgcaagcagcggtggtgacggggatgaacagttctttggccctggaaccagactcaccgtgctcgaggacctcaagaacgtgttcccacccgaagtcgcggtgttcgagccctccaaggcggagatcgcccatactcagaaagccactctcgtgtgcctggccaccggattctacccggaccacgtcgagctctcttggtgggtgaacgggaaagaggtccacagcggcgtgagcactgatccgcagccgctgaaggaacaacccgccttgaacgactcgcggtactgtctgtcctcccggctgagagtgtcggccaccttctggcaaaaccccaggaaccactttaggtgccaagtccagttctacggcctgagcgaaaacgatgagtggacccaggacagagccaagcctgtgacccagattgtgtcagccgaggcttggggtagagcagactgcggaatcaccagcgccagctaccaccaaggcgtcctctcggcgaccattctgtacgaaatcctgcttgggaaggccactctgtacgccgtgctggtgtccgccctggtgctgatggccatggtcaagcggaaggactcccgggggagagcaaagaggggatcgggagccaccaattttagcctgctgaagcaggccggcgatgtggaagaaaatcctggccccatgtcccttagctcactgctgaaagtggtcactgcgagcctgtggctgggaccaggcattgctcaaaagatcacccagactcagcctgggatgttcgtgcaagagaaggaagccgtgaccctcgactgcacttacgacacctccgacccgtcctacgggctgttctggtacaagcagccgtcctccggagagatgatcttcctcatctaccaaggctcctatgatcagcagaacgccaccgaaggacgctacagcctgaacttccagaaggctcggaagtcggcgaacctcgtgatcagcgcatcccaactgggggacagcgccatgtacttctgtgccatgtcgggcggatacaccgggggattcaagaccattttcggggccggcactagactgttcgtgaaggccaacatccagaatcctgatccggcggtgtatcagctgcgcgactccaagtcttccgataaatccgtgtgtctctttacagacttcgactcccaaaccaacgtgtcacagtccaaggacagcgatgtgtacatcaccgacaaaaccgtgctggacatgcggtccatggacttcaagtcaaacagcgcagtcgcctggtccaacaagtccgacttcgcctgtgcgaacgccttcaacaactccatcattccggaagatacctttttcccttcaagcgacgtcccctgtgatgtgaagctcgtggaaaagtcgtttgaaacggacaccaacctgaactttcagaacctgctagtgattgtgctccgcatcctgctgctgaaggtcgccggcttcaacttgctgatgacgctccggctgtggtcctcgtaa

SEQ ID NO: 108 - protein, 277 aa, Artificial Sequence
  TCR-8 a complete
MSLSSLLKVVTASLWLGPGIAQKITQTQPGMFVQEKEAVTLDCTYDTSDPSYGLFWYKQPSSGEMIFLIYQGSYDQQNATEGRYSLNFQKARKSANLVISASQLGDSAMYFCAMSGGYTGGFKTIFGAGTRLFVKANIQNPDPAVYQLRDSKSSDKSVCLFTDFDSQTNVSQSKDSDVYITDKTVLDMRSMDFKSNSAVAWSNKSDFACANAFNNSIIPEDTFFPSSDVPCDVKLVEKSFETDTNLNFQNLLVIVLRILLLKVAGFNLLMTLRLWSS

SEQ ID NO: 109 - protein, 310 aa, Artificial Sequence
  TCR-8 b complete
MGFRLLCCVAFCLLGAGPVDSGVTQTPKHLITATGQRVTLRCSPRSGDLSVYWYQQSLDQGLQFLIQYYNGEERAKGNILERFSAQQFPDLHSELNLSSLELGDSALYFCASSGGDGDEQFFGPGTRLTVLEDLKNVFPPEVAVFEPSKAEIAHTQKATLVCLATGFYPDHVELSWWVNGKEVHSGVSTDPQPLKEQPALNDSRYCLSSRLRVSATFWQNPRNHFRCQVQFYGLSENDEWTQDRAKPVTQIVSAEAWGRADCGITSASYHQGVLSATILYEILLGKATLYAVLVSALVLMAMVKRKDSRG

SEQ ID NO: 110 - protein, 613 aa, Artificial Sequence
  TCR-8 polyprotein
MGFRLLCCVAFCLLGAGPVDSGVTQTPKHLITATGQRVTLRCSPRSGDLSVYWYQQSLDQGLQFLIQYYNGEERAKGNILERFSAQQFPDLHSELNLSSLELGDSALYFCASSGGDGDEQFFGPGTRLTVLEDLKNVFPPEVAVFEPSKAEIAHTQKATLVCLATGFYPDHVELSWWVNGKEVHSGVSTDPQPLKEQPALNDSRYCLSSRLRVSATFWQNPRNHFRCQVQFYGLSENDEWTQDRAKPVTQIVSAEAWGRADCGITSASYHQGVLSATILYEILLGKATLYAVLVSALVLMAMVKRKDSRGRAKRGSGATNFSLLKQAGDVEENPGPMSLSSLLKVVTASLWLGPGIAQKITQTQPGMFVQEKEAVTLDCTYDTSDPSYGLFWYKQPSSGEMIFLIYQGSYDQQNATEGRYSLNFQKARKSANLVISASQLGDSAMYFCAMSGGYTGGFKTIFGAGTRLFVKANIQNPDPAVYQLRDSKSSDKSVCLFTDFDSQTNVSQSKDSDVYITDKTVLDMRSMDFKSNSAVAWSNKSDFACANAFNNSIIPEDTFFPSSDVPCDVKLVEKSFETDTNLNFQNLLVIVLRILLLKVAGFNLLMTLRLWSS

SEQ ID NO: 111 - DNA, 819 bp, Artificial Sequence
  TCR-9 a complete
atgacgtccattagagccgtgttcattttcctgtggctgcaactggacctcgtgaatggagaaaacgtcgagcagcacccatccaccctgagcgtgcaggagggagactccgcagtcatcaagtgcacttactccgactcagcatcaaactatttcccgtggtataagcaggaactcggaaagcggcctcagctcatcattgacatccgctccaacgtcggagagaagaaggaccagagaattgccgtgacactcaacaagaccgccaagcatttctcccttcacatcaccgaaacccagcccgaggacagcgccgtctacttttgtgcggcctcgaggggcactgggtttcagaagctcgtgttcggcactgggacccggctgctggtgtcgccaaacatccagaatccagaccccgcggtgtaccagctgagagactcgaagtcttccgataaatccgtgtgtctctttacagacttcgatagccagactaacgtgtcccagtccaaggactccgatgtgtacatcaccgacaagactgtgctggatatgcggagcatggactttaagtccaattcagcggtcgcgtggagcaacaagtccgacttcgcctgcgctaacgctttcaacaactccattatcccggaggataccttcttcccgtcaagcgacgtcccctgcgacgtgaagctggtcgagaagtccttcgaaaccgataccaacctgaacttccaaaacctcctagtgattgtgctcagaatcctgctgctgaaagtggctggcttcaatttgctgatgaccctgcggctctggagcagc

SEQ ID NO: 112 - DNA, 930 bp, Artificial Sequence
  TCR-9 b complete
atgggttgtcggttgctgtgttgcgtcgtgttctgccttcttcaagctggtcctctcgatactgccgtgagccaaacccctaagtaccttgtcacccaaatgggcaacgacaagtccatcaaatgcgaacagaacctcggacacgacaccatgtactggtacaaacaggattccaagaagttcctgaagattatgttctcatacaacaacaaggaactgattatcaacgaaactgtgccgaaccggttctcaccgaagtcgcctgacaaggctcatctcaacttgcatatcaactcgctggagctcggcgactccgccgtgtacttctgcgcgtccagccagttctgggacggagcgggcgacgaacagtacttcggcccgggcactcggctgaccgtgaccgaagatctgaacaaagtgttcccccccgaagtggccgtgttcgaaccttccaaggcggagatcgcccacacccaaaaggccactctggtctgcctggccaccggtttcttccccgatcacgtggaactgtcttggtgggtgaacggaaaagaagtgcactcgggggtgtccacggacccccagcctctgaaggaacagccggcactgaatgactcacgctactgtctgtcgtcacggctgcgcgtgtcggccaccttctggcaaaacccgcgaaaccactttcgctgccaagtgcagttttacgggctttccgagaacgacgagtggactcaggacagagcgaagcccgtgacccaaatcgtgtccgccgaggcctggggacgcgccgactgcggtatcaccagcgccagctaccaccagggcgtgctgtcagctaccatcctttacgagatcctcctgggaaaggccaccctctacgccgtcctggtgtccgcactggtgctgatggctatggtcaagcggaaggat

SEQ ID NO: 113 - DNA, 1833 bp, Artificial Sequence
  TCR-9 polycistronic construct
atgggttgtcggttgctgtgttgcgtcgtgttctgccttcttcaagctggtcctctcgatactgccgtgagccaaacccctaagtaccttgtcacccaaatgggcaacgacaagtccatcaaatgcgaacagaacctcggacacgacaccatgtactggtacaaacaggattccaagaagttcctgaagattatgttctcatacaacaacaaggaactgattatcaacgaaactgtgccgaaccggttctcaccgaagtcgcctgacaaggctcatctcaacttgcatatcaactcgctggagctcggcgactccgccgtgtacttctgcgcgtccagccagttctgggacggagcgggcgacgaacagtacttcggcccgggcactcggctgaccgtgaccgaagatctgaacaaagtgttcccccccgaagtggccgtgttcgaaccttccaaggcggagatcgcccacacccaaaaggccactctggtctgcctggccaccggtttcttccccgatcacgtggaactgtcttggtgggtgaacggaaaagaagtgcactcgggggtgtccacggacccccagcctctgaaggaacagccggcactgaatgactcacgctactgtctgtcgtcacggctgcgcgtgtcggccaccttctggcaaaacccgcgaaaccactttcgctgccaagtgcagttttacgggctttccgagaacgacgagtggactcaggacagagcgaagcccgtgacccaaatcgtgtccgccgaggcctggggacgcgccgactgcggtatcaccagcgccagctaccaccagggcgtgctgtcagctaccatcctttacgagatcctcctgggaaaggccaccctctacgccgtcctggtgtccgcactggtgctgatggctatggtcaagcggaaggattttagggccaaacgcgggtccggagcgaccaacttctcgctgttgaagcaggccggcgatgtggaagagaaccctggaccgatgacgtccattagagccgtgttcattttcctgtggctgcaactggacctcgtgaatggagaaaacgtcgagcagcacccatccaccctgagcgtgcaggagggagactccgcagtcatcaagtgcacttactccgactcagcatcaaactatttcccgtggtataagcaggaactcggaaagcggcctcagctcatcattgacatccgctccaacgtcggagagaagaaggaccagagaattgccgtgacactcaacaagaccgccaagcatttctcccttcacatcaccgaaacccagcccgaggacagcgccgtctacttttgtgcggcctcgaggggcactgggtttcagaagctcgtgttcggcactgggacccggctgctggtgtcgccaaacatccagaatccagaccccgcggtgtaccagctgagagactcgaagtcttccgataaatccgtgtgtctctttacagacttcgatagccagactaacgtgtcccagtccaaggactccgatgtgtacatcaccgacaagactgtgctggatatgcggagcatggactttaagtccaattcagcggtcgcgtggagcaacaagtccgacttcgcctgcgctaacgctttcaacaactccattatcccggaggataccttcttcccgtcaagcgacgtcccctgcgacgtgaagctggtcgagaagtccttcgaaaccgataccaacctgaacttccaaaacctcctagtgattgtgctcagaatcctgctgctgaaagtggctggcttcaatttgctgatgaccctgcggctctggagcagctaa

SEQ ID NO: 114 - protein, 273 aa, Artificial Sequence
  TCR-9 a complete
MTSIRAVFIFLWLQLDLVNGENVEQHPSTLSVQEGDSAVIKCTYSDSASNYFPWYKQELGKRPQLIIDIRSNVGEKKDQRIAVTLNKTAKHFSLHITETQPEDSAVYFCAASRGTGFQKLVFGTGTRLLVSPNIQNPDPAVYQLRDSKSSDKSVCLFTDFDSQTNVSQSKDSDVYITDKTVLDMRSMDFKSNSAVAWSNKSDFACANAFNNSIIPEDTFFPSSDVPCDVKLVEKSFETDTNLNFQNLLVIVLRILLLKVAGFNLLMTLRLWSS

SEQ ID NO: 115 - protein, 310 aa, Artificial Sequence
  TCR-9 b complete
MGCRLLCCVVFCLLQAGPLDTAVSQTPKYLVTQMGNDKSIKCEQNLGHDTMYWYKQDSKKFLKIMFSYNNKELIINETVPNRFSPKSPDKAHLNLHINSLELGDSAVYFCASSQFWDGAGDEQYFGPGTRLTVTEDLNKVFPPEVAVFEPSKAEIAHTQKATLVCLATGFFPDHVELSWWVNGKEVHSGVSTDPQPLKEQPALNDSRYCLSSRLRVSATFWQNPRNHFRCQVQFYGLSENDEWTQDRAKPVTQIVSAEAWGRADCGITSASYHQGVLSATILYEILLGKATLYAVLVSALVLMAMVKRKD

SEQ ID NO: 116 - protein, 610 aa, Artificial Sequence
  TCR-9 polyprotein
MGCRLLCCVVFCLLQAGPLDTAVSQTPKYLVTQMGNDKSIKCEQNLGHDTMYWYKQDSKKFLKIMFSYNNKELIINETVPNRFSPKSPDKAHLNLHINSLELGDSAVYFCASSQFWDGAGDEQYFGPGTRLTVTEDLNKVFPPEVAVFEPSKAEIAHTQKATLVCLATGFFPDHVELSWWVNGKEVHSGVSTDPQPLKEQPALNDSRYCLSSRLRVSATFWQNPRNHFRCQVQFYGLSENDEWTQDRAKPVTQIVSAEAWGRADCGITSASYHQGVLSATILYEILLGKATLYAVLVSALVLMAMVKRKDFRAKRGSGATNFSLLKQAGDVEENPGPMTSIRAVFIFLWLQLDLVNGENVEQHPSTLSVQEGDSAVIKCTYSDSASNYFPWYKQELGKRPQLIIDIRSNVGEKKDQRIAVTLNKTAKHFSLHITETQPEDSAVYFCAASRGTGFQKLVFGTGTRLLVSPNIQNPDPAVYQLRDSKSSDKSVCLFTDFDSQTNVSQSKDSDVYITDKTVLDMRSMDFKSNSAVAWSNKSDFACANAFNNSIIPEDTFFPSSDVPCDVKLVEKSFETDTNLNFQNLLVIVLRILLLKVAGFNLLMTLRLWSS